European Patent Specification EP 3 501 519 B1, published November 20, 2024. Title: Immunomodulators. Applicant: Nara Institute of Science and Technology. The sequence listing filed with the application follows.

SEQUENCE LISTING (4 sequences)

SEQ ID NO: 1 - DNA, 20 bp, Artificial Sequence
  synthetic oligonucleotide
cctggctgttcccctatgaa

SEQ ID NO: 2 - DNA, 21 bp, Artificial Sequence
  synthetic oligonucleotide
gagctggtgggagtgtcagtg

SEQ ID NO: 3 - DNA, 20 bp, Artificial Sequence
  synthetic oligonucleotide
gggagtcaagaaagtcacgc

SEQ ID NO: 4 - DNA, 20 bp, Artificial Sequence
  synthetic oligonucleotide
ggctttgaaagttctttcac